European Patent Specification EP 3 746 791 B1, published March 6, 2024. Title: Use of BMMF Rep Protein as Biomarker for Colon Cancer. Applicant: Deutsches Krebsforschungszentrum. The sequence listing filed with the application follows.

SEQUENCE LISTING (19 sequences)

SEQ ID NO: 1 - protein, 324 aa, artificial sequence
  MSBI1 Rep protein
MSDLIVKDNALMNASYNLALVEQRLILLAIIEARETGKGINANDPLTVHASSYINQFNVERHTAYQALKDACKDLFARQFSYQEKRERGRINITSRWVSQIGYMDDTATVEIIFAPAVVPLITRLEEQFTQYDIEQISGLSSAYAVRMYELLICWRSTGKTPIIELDEFRKRIGVLDTEYTRTDNLKMRVIELALKQINEHTDITASYEQHKKGRVITGFSFKFKHKKQNSDKTPKNSDSSPRIVKHSQIPTNIVKQPENAKMSDLEHRASRVTGEIMRNRLSDRFKQGDESAIDMMKRIQSEIITDAIADQWESKLEEFGVVF

SEQ ID NO: 2 - protein, 18 aa, artificial sequence
  Rep peptide
EARETGKGINANDPLTVH

SEQ ID NO: 3 - protein, 20 aa, artificial sequence
  Rep peptide
KQINEHTDITASYEHKKGRT

SEQ ID NO: 4 - protein, 8 aa, artificial sequence
  His tag
GAHHHHHH

SEQ ID NO: 5 - protein, 11 aa, artificial sequence
  T7 tag
MASMTGGQQMG

SEQ ID NO: 6 - protein, 8 aa, artificial sequence
  FLAG tag
DYKDDDDK

SEQ ID NO: 7 - protein, 8 aa, artificial sequence
  Trep II tag
WSHPQFEK

SEQ ID NO: 8 - protein, 319 aa, artificial sequence
  MSBI2.176
MSKLVVKDNALMNASYNLDLVEQRLILLAIIEARESGKGINANDPLTVHAESYINQFGVHRVTAYQALKDACDNLFARQFSYQSKSEKGNIQNHRSRWVSEIIYIDTEATVKIIFAPAIVPLITRLEEQFTKYDIEQISDLSSAYAIRLYELLICWRSTGKTPIIGLGEFRNRVGVLDSEYHRIAHLKERVIEHSIKQINEHTDITATYEQHKKGRTITGFSFKFKQKKPKQAEIATETPKTATNDPDTTKPLTEPQIAKYSMILCKLGSISDLSNFPDYPAFANWIGNILRNPEKADEQIAKRIFTALKTETDYSKKN

SEQ ID NO: 9 - protein, 7 aa, artificial sequence
  MSBI1 epitope
NRLSDRF

SEQ ID NO: 10 - protein, 326 aa, Artificial Sequence
  CMI1.252
MSDLIVKDNALMNASYNLALVEQRLILLAILEARETGKGINANDPLTVHASSYINQFNVERHTAYQALKDACKDLFARQFSYQEKRERGRINITSRWVSQIGYMDDTATVEIIFAPAVVPLITRLEEQFTQYDIEQISELSSAYAVRLYELLICWRSTGKTPIIDLTEFRKRLGVLDTEYTRTDNLKMRVIELGLKQINEHTDITASYEQHKKGRTITGFSFKFKQKKKTGAEMPKNSDSSPHIEKPSQIPANIAKQPENAKKDDLGHRASKITGLIMSNGLADRFKRGDESVIDMMKRIKEEITTDTTADQWENKLEEFGVIFQS

SEQ ID NO: 11 - protein, 324 aa, Artificial Sequence
  CMI2.214
MSDLIVKDNALMNASYNLDLVEQRLILLAILEARETGKGINANDPLTVHAESYINQFGVARQTAYQALKDACKDLFARQFSYQEKRERGRANITSRWVSQIAYIDETATVEVIFAPAVVPLITRLEEQFTQYDIEQISGLSSAYAVRLYELLICWRSTGKTPVIELAEFRKRLGVLNDEYTRSDNFKKWIIENPIKQINEHTDITASYEQHKKGRTITGFSFKFKQKKKTEPETPKNSDSSQRIEKPSQIPANIVKQPENANLSDLQHRASKITGLIMSNRLSDRFKQGDESIMQMMARIQSEITTDSIADQWQSKLEEFGVVF

SEQ ID NO: 12 - protein, 324 aa, Artificial Sequence
  CMI3.168
MSDLIVKDNALMNASYNLALVEQRLILLAILEARETGKGINANDPLTVHASSYINQFNVERHTAYQALKDACKDLFARQFSYQEKRERGRANITSRWVSQIAYIDETATVEVIFAPAVVPLITRLEEQFTQYDIEQISGLSSAYAVRLYELLICWRTTGKTPVLDLTEFRKRLGVLDTEYTRTDNLKMRVIEQSLKQINKHTDITASYEQHKKGRTITGFSFKFKQKKKTEPETPKNNDSGVSKPKTVEIPAEVVKQPKNTNLSDLEKRVRMITGAIAKNNLASRFQHGNESPLDMMKRIQSEITSDETADLWQNKLESMGVVF

SEQ ID NO: 13 - DNA, 999 bp, artificial sequence
  codon-optimized MSBI1
atgagcgacctgatcgtgaaagacaatgccctgatgaacgcctcctacaacctggcactggtcgaacagagactgattctgctggctatcatcgaggcaagggagaccggcaagggcatcaacgccaatgaccccctgacagtgcacgccagctcctacatcaaccagtttaatgtggagcgccacaccgcctatcaggccctgaaggacgcctgcaaggatctgtttgcccggcagttcagctaccaggagaagcgggagagaggcaggatcaacatcacaagcagatgggtgtcccagatcggctatatggacgataccgccacagtggagatcatctttgcaccagcagtggtgcctctgatcaccaggctggaggagcagttcacacagtacgacatcgagcagatctccggactgtctagcgcctacgccgtgcgcatgtatgagctgctgatctgttggcggtctaccggcaagacacctatcatcgagctggatgagttccgcaagcggatcggcgtgctggacaccgagtacaccagaacagataacctgaagatgagagtgatcgagctggccctgaagcagatcaatgagcacaccgatatcacagcctcttatgagcagcacaagaagggccgcgtgatcaccggcttcagctttaagttcaagcacaagaagcagaactctgacaagacaccaaagaatagcgattcctctccccggatcgtgaagcacagccagatccctaccaacatcgtgaagcagccagagaatgccaagatgtccgacctggagcacagggcatctagggtgacaggcgagatcatgagaaataggctgagcgatcggttcaagcagggcgacgagtccgccatcgatatgatgaagagaatccagtccgagatcatcaccgacgccatcgccgatcagtgggaatctaaactggaagagtttggagtcgtgtttggagcacatcaccatcatcatcactga

SEQ ID NO: 14 - protein, 326 aa, artificial sequence
  MSBI1 protein
MSDLIVKDNALMNASYNLALVEQRLILLAIIEARETGKGINANDPLTVHASSYINQFNVERHTAYQALKDACKDLFARQFSYQEKRERGRINITSRWVSQIGYMDDTATVEIIFAPAVVPLITRLEEQFTQYDIEQISGLSSAYAVRMYELLICWRSTGKTPIIELDEFRKRIGVLDTEYTRTDNLKMRVIELALKQINEHTDITASYEQHKKGRVITGFSFKFKHKKQNSDKTPKNSDSSPRIVKHSQIPTNIVKQPENAKMSDLEHRASRVTGEIMRNRLSDRFKQGDESAIDMMKRIQSEIITDAIADQWESKLEEFGVVFGA

SEQ ID NO: 15 - DNA, 974 bp, artificial sequence
  MSBI1 wild type
atgagcgatttaatagtaaaagataacgccctaatgaatgctagttataacttagctttggttgaacagaggttaattctattagcaatcatagaagcgagagaaacaggcaaagggattaatgccaatgatcctttaacagttcatgcaagtagctatatcaatcaatttaacgtagaaaggcatacggcatatcaagccctcaaagatgcttgtaaagacttgtttgcccgtcaattcagttaccaagaaaagcgagaacgaggacgaattaatattacaagtcgatgggtttcgcaaattggctatatggacgatacagcaaccgttgagattatttttgcccctgcggttgttcctctgattacacggctagaggaacagttcacccagtacgatattgagcaaattagcggtttatcgagtgcatatgctgttcgtatgtacgaactgctgatttgttggcgtagcacaggcaaaacaccaattattgagctagacgagtttagaaagcgaataggtgttttagatactgaatacactagaacagataatttaaagatgcgagttattgaattagccctaaaacaaatcaacgaacatacagacatcacagcaagctatgaacaacacaaaaaagggcgagtgattacaggattctcattcaagtttaagcacaagaaacaaaacagcgataaaacgccaaaaaatagcgattctagcccacgtatcgtaaaacatagtcaaatccctccaacattgtaaaacagcctgaaaacgccaaaatgagcgatttagaacatagagcgagccgtgttacaggggaaataatgcgaaatcgtctgtcagatcggtttaaacaaggcgatgaatcagcaatcgacatgatgaaacgtattcaaagtgaaataataaccgatgcaatagcagaccagtgggaaagcaaactggaggagtttggcgtggttttttag

SEQ ID NO: 16 - DNA, 24 bp, Artificial Sequence
  primer
gaggacgaattaatattacaagtc

SEQ ID NO: 17 - DNA, 20 bp, Artificial Sequence
  primer
gttctcgcttttcttggtaa

SEQ ID NO: 18 - DNA, 19 bp, Artificial Sequence
  primer
ggattaatgccaatgatcc

SEQ ID NO: 19 - DNA, 18 bp, Artificial Sequence
  primer
ctttgcctgtttctctcg